European Patent Application EP 4 745 154 A1, published May 20, 2026. Title: 一种分离的TCR及其用途. Applicant: 上海市第一人民医院. Application CN. The sequence listing filed with the application follows.

SEQUENCE LISTING (15 sequences)

SEQ ID NO: 1 - protein, 15 aa, synthetic construct
CASSDDTGANYGYTF

SEQ ID NO: 2 - protein, 12 aa, synthetic construct
CAPDNAGNMLTF

SEQ ID NO: 3 - protein, 6 aa, synthetic construct
NYSPAY

SEQ ID NO: 4 - protein, 7 aa, synthetic construct
IRENEKE

SEQ ID NO: 5 - protein, 5 aa, synthetic construct
SNHLY

SEQ ID NO: 6 - protein, 6 aa, synthetic construct
FYNNEI

SEQ ID NO: 7 - protein, 307 aa, synthetic construct
MDTWLVCWAIFSLLKAGLTEPEVTQTPSHQVTQMGQEVILRCVPISNHLYFYWYRQILGQKVEFLVSFYNNEISEKSEIFDDQFSVERPDGSNFTLKIRSTKLEDSAMYFCASSDDTGANYGYTFGSGTRLTVVEDLRNVTPPKVSLFEPSKAEIANKQKATLVCLARGFFPDHVELSWWVNGKEVHSGVCTDPQAYKESNYSYCLSSRLRVSATFWHNPRNHFRCQVQFHGLSEEDKWPEGSPKPVTQNISAEAWGRADCGITSASYQQGVLSATILYEILLGKATLYAVLVSTLVVMAMVKRKNS

SEQ ID NO: 8 - protein, 268 aa, synthetic construct
MESFLGGVLLILWLQVDWVKSQKIEQNSEALNIQEGKTATLTCNYTNYSPAYLQWYRQDPGRGPVFLLLIRENEKEKRKERLKVTFDTTLKQSLFHITASQPADSATYLCAPDNAGNMLTFGGGTRLMVKPHIQNPEPAVYQLKDPRSQDSTLCLFTDFDSQINVPKTMESGTFITDKCVLDMKAMDSKSNGAIAWSNQTSFTCQDIFKETNATYPSSDVPCDATLTEKSFETDMNLNFQNLSVMGLRILLLKVAGFNLLMTLRLWSS

SEQ ID NO: 9 - DNA, 1725 bp, synthetic construct
  source 1..1725: mol_type = other DNA
atggagagcttcctgggcggcgtgctgctgatcctgtggctgcaggtggactgggtgaagagccagaagatcgagcagaacagcgaggccctgaacatccaggagggcaagaccgccaccctgacctgcaactacaccaactacagccccgcctacctgcagtggtacaggcaggaccccggcaggggccccgtgttcctgctgctgatcagggagaacgagaaggagaagaggaaggagaggctgaaggtgaccttcgacaccaccctgaagcagagcctgttccacatcaccgccagccagcccgccgacagcgccacctacctgtgcgcccccgacaacgccggcaacatgctgaccttcggcggcggcaccaggctgatggtgaagccccacatccagaaccccgagcccgccgtgtaccagctgaaggaccccaggagccaggacagcaccctgtgcctgttcaccgacttcgacagccagatcaacgtgcccaagaccatggagagcggcaccttcatcaccgacaagtgcgtgctggacatgaaggccatggacagcaagagcaacggcgccatcgcctggagcaaccagaccagcttcacctgccaggacatcttcaaggagaccaacgccacctaccccagcagcgacgtgccctgcgacgccaccctgaccgagaagagcttcgagaccgacatgaacctgaacttccagaacctgagcgtgatgggcctgaggatcctgctgctgaaggtggccggcttcaacctgctgatgaccctgaggctgtggagcagcatggacacctggctggtgtgctgggccatcttcagcctgctgaaggccggcctgaccgagcccgaggtgacccagacccccagccaccaggtgacccagatgggccaggaggtgatcctgaggtgcgtgcccatcagcaaccacctgtacttctactggtacaggcagatcctgggccagaaggtggagttcctggtgagcttctacaacaacgagatcagcgagaagagcgagatcttcgacgaccagttcagcgtggagaggcccgacggcagcaacttcaccctgaagatcaggagcaccaagctggaggacagcgccatgtacttctgcgccagcagcgacgacaccggcgccaactacggctacaccttcggcagcggcaccaggctgaccgtggtggaggacctgaggaacgtgaccccccccaaggtgagcctgttcgagcccagcaaggccgagatcgccaacaagcagaaggccaccctggtgtgcctggccaggggcttcttccccgaccacgtggagctgagctggtgggtgaacggcaaggaggtgcacagcggcgtgtgcaccgacccccaggcctacaaggagagcaactacagctactgcctgagcagcaggctgagggtgagcgccaccttctggcacaaccccaggaaccacttcaggtgccaggtgcagttccacggcctgagcgaggaggacaagtggcccgagggcagccccaagcccgtgacccagaacatcagcgccgaggcctggggcagggccgactgcggcatcaccagcgccagctaccagcagggcgtgctgagcgccaccatcctgtacgagatcctgctgggcaaggccaccctgtacgccgtgctggtgagcaccctggtggtgatggccatggtgaagaggaagaacagc

SEQ ID NO: 10 - protein, 173 aa, synthetic construct
EDLRNVTPPKVSLFEPSKAEIANKQKATLVCLARGFFPDHVELSWWVNGKEVHSGVCTDPQAYKESNYSYCLSSRLRVSATFWHNPRNHFRCQVQFHGLSEEDKWPEGSPKPVTQNISAEAWGRADCGITSASYQQGVLSATILYEILLGKATLYAVLVSTLVVMAMVKRKNS

SEQ ID NO: 11 - protein, 137 aa, synthetic construct
DIQNPEPAVYQLKDPRSQDSTLCLFTDFDSQINVPKTMESGTFITDKCVLDMKAMDSKSNGAIAWSNQTSFTCQDIFKETNATYPSSDVPCDATLTEKSFETDMNLNFQNLSVMGLRILLLKVAGFNLLMTLRLWSS

SEQ ID NO: 12 - DNA, 1725 bp, synthetic construct
  source 1..1725: mol_type = other DNA
atggaatctttccttggaggagtactgctcattttgtggctgcaagtcgactgggtgaaaagtcagaagatcgaacagaatagcgaagccctgaacatccaggaaggcaagactgctacactgacttgtaactacacaaactatagcccagcgtacctgcagtggtaccggcaggatcccggaagaggccccgtgttcctgctgcttatcagagaaaacgaaaaggaaaaacgaaaggagcggctgaaggttacatttgataccacccttaaacagtccctgtttcacattactgcaagtcagccagctgactccgcaacatatctgtgcgcccccgacaacgcgggtaatatgcttacgtttggcggaggtaccagacttatggtaaagccgcacatccagaatcctgagcctgcggtttaccagttgaaagatccaaggtcacaggactccacattgtgcctgttcacagacttcgattcccagatcaatgtgcctaagacgatggagtccggaacctttattacggacaaatgcgtgctggatatgaaggcgatggatagcaagtcaaacggcgcaatcgcttggtcaaaccagacaagcttcacctgtcaggatatattcaaagagactaacgcaacctatccctcttcagatgtaccatgcgacgctactttgaccgaaaagtctttcgaaaccgacatgaacctgaacttccagaacctttcagtgatgggacttcgcattttgctgcttaaagttgctggctttaatctgcttatgacattgcggctttggtcctctatggatacttggctggtatgctgggccatattcagtctgctcaaagccggacttaccgaacctgaagtgacacaaactcccagccaccaagtgactcagatgggccaggaggtaatcttgaggtgtgtgcctatctccaatcacttgtacttctactggtaccgccaaattttggggcaaaaagtggagtttctggtgagcttttataacaacgagatctctgaaaaatctgagatcttcgacgatcagttttcagtggagcgacccgatggaagcaactttacgcttaaaattcgcagtacgaagctggaagacagcgcaatgtatttttgcgcgagcagtgatgataccggcgccaattacggttacacattcggcagcggcacccgcctcaccgtggtggaggaccttaggaacgtgacacctcctaaggtgagcttgtttgagcccagtaaagcagagattgccaataagcagaaggctaccctcgtttgcctcgcccggggattctttcccgaccatgttgaactgagctggtgggtgaatgggaaggaagttcatagcggggtgtgtaccgatccacaagcatacaaagagagcaactacagctattgtctgtcttccaggctccgcgtcagtgctacgttctggcacaaccctcggaatcatttcaggtgtcaggttcagtttcacggactgtccgaagaggataaatggcctgaaggaagtcctaagcctgttacccagaatattagcgccgaagcttggggcagggcagactgcggaatcactagcgcctcataccagcaaggcgtgctgtccgctacaattctttatgagatcctcttggggaaggccaccctgtatgctgtgcttgtgagtacactggtcgttatggccatggtgaagcgaaaaaattct

SEQ ID NO: 13 - DNA, 1803 bp, synthetic construct
  source 1..1803: mol_type = other DNA
atggacacctggctggtgtgctgggccatcttcagcctgctgaaggccggcctgaccgagcccgaggtgacccagacccccagccaccaggtgacccagatgggccaggaggtgatcctgaggtgcgtgcccatcagcaaccacctgtacttctactggtacaggcagatcctgggccagaaggtggagttcctggtgagcttctacaacaacgagatcagcgagaagagcgagatcttcgacgaccagttcagcgtggagaggcccgacggcagcaacttcaccctgaagatcaggagcaccaagctggaggacagcgccatgtacttctgcgccagcagcgacgacaccggcgccaactacggctacaccttcggcagcggcaccaggctgaccgtggtggaggacctgaggaacgtgaccccccccaaggtgagcctgttcgagcccagcaaggccgagatcgccaacaagcagaaggccaccctggtgtgcctggccaggggcttcttccccgaccacgtggagctgagctggtgggtgaacggcaaggaggtgcacagcggcgtgtgcaccgacccccaggcctacaaggagagcaactacagctactgcctgagcagcaggctgagggtgagcgccaccttctggcacaaccccaggaaccacttcaggtgccaggtgcagttccacggcctgagcgaggaggacaagtggcccgagggcagccccaagcccgtgacccagaacatcagcgccgaggcctggggcagggccgactgcggcatcaccagcgccagctaccagcagggcgtgctgagcgccaccatcctgtacgagatcctgctgggcaaggccaccctgtacgccgtgctggtgagcaccctggtggtgatggccatggtgaagaggaagaacagcagggccaagaggggcagcggcgccaccaacttcagcctgctgaagcaggccggcgacgtggaggagaaccccggccccatggagagcttcctgggcggcgtgctgctgatcctgtggctgcaggtggactgggtgaagagccagaagatcgagcagaacagcgaggccctgaacatccaggagggcaagaccgccaccctgacctgcaactacaccaactacagccccgcctacctgcagtggtacaggcaggaccccggcaggggccccgtgttcctgctgctgatcagggagaacgagaaggagaagaggaaggagaggctgaaggtgaccttcgacaccaccctgaagcagagcctgttccacatcaccgccagccagcccgccgacagcgccacctacctgtgcgcccccgacaacgccggcaacatgctgaccttcggcggcggcaccaggctgatggtgaagcccgacatccagaaccccgagcccgccgtgtaccagctgaaggaccccaggagccaggacagcaccctgtgcctgttcaccgacttcgacagccagatcaacgtgcccaagaccatggagagcggcaccttcatcaccgacaagtgcgtgctggacatgaaggccatggacagcaagagcaacggcgccatcgcctggagcaaccagaccagcttcacctgccaggacatcttcaaggagaccaacgccacctaccccagcagcgacgtgccctgcgacgccaccctgaccgagaagagcttcgagaccgacatgaacctgaacttccagaacctgagcgtgatgggcctgaggatcctgctgctgaaggtggccggcttcaacctgctgatgaccctgaggctgtggagcagc

SEQ ID NO: 14 - protein, 131 aa, synthetic construct
MESFLGGVLLILWLQVDWVKSQKIEQNSEALNIQEGKTATLTCNYTNYSPAYLQWYRQDPGRGPVFLLLIRENEKEKRKERLKVTFDTTLKQSLFHITASQPADSATYLCAPDNAGNMLTFGGGTRLMVKP

SEQ ID NO: 15 - protein, 134 aa, synthetic construct
MDTWLVCWAIFSLLKAGLTEPEVTQTPSHQVTQMGQEVILRCVPISNHLYFYWYRQILGQKVEFLVSFYNNEISEKSEIFDDQFSVERPDGSNFTLKIRSTKLEDSAMYFCASSDDTGANYGYTFGSGTRLTVV